European Patent Specification EP 3 728 610 B1, published May 31, 2023. Title: Constructs comprising neuronal viability factors and uses thereof. Applicant: SparingVision et al. The sequence listing filed with the application follows.

SEQUENCE LISTING (16 sequences)

SEQ ID NO: 1 - protein, 109 aa, Homo sapiens
MASLFSGRILIRNNSDQDELDTEAEVSRRLENRLVLLFFGAGACPQCQAFVPILKDFFVRLTDEFYVLRAAQLALVYVSQDSTEEQQDLFLKDMPKKWLFLPFEDDLRR

SEQ ID NO: 2 - protein, 212 aa, Homo sapiens
MASLFSGRILIRNNSDQDELDTEAEVSRRLENRLVLLFFGAGACPQCQAFVPILKDFFVRLTDEFYVLRAAQLALVYVSQDSTEEQQDLFLKDMPKKWLFLPFEDDLRRDLGRQFSVERLPAVVVLKPDGDVLTRDGADEIQRLGTACFANWQEAAEVLDRNFQLPEDLEDQEPRSLTECLRRHKYRVEKAARGGRDPGGGGGEEGGAGGLF

SEQ ID NO: 3 - DNA, 330 bp, Homo sapiens
atggcctccctgttctctggccgcatcctgatccgcaacaatagcgaccaggacgagctggatacggaggctgaggtcagtcgcaggctggagaaccggctggtgctgctgttctttggtgctggggcttgtccacagtgccaggccttcgtgcccatcctcaaggacttcttcgtgcggctcacagatgagttctatgtactgcgggcggctcagctggccctggtgtacgtgtcccaggactccacggaggagcagcaggacctgttcctcaaggacatgccaaagaaatggcttttcctgccctttgaggatgatctgaggaggtga

SEQ ID NO: 4 - DNA, 330 bp, Pan troglodytes
atggcctccctgttctctggccgcatcctgatccgcaacaatagcgaccaggacgaactggatacggaggctgaggtcagtcgcaggctggagaaccggctggtgctgctgttctttggtgccggggcttgtccacagtgccaggccttcgtgcccatcctcaaggacttcttcgtgcggctcacagatgagttctatgtactgcgggcggctcagctggccctggtgtacgtgtcccaggactccacggaggagcagcaggacctgttcctcaaggacatgccaaagaagtggcttttcctgccctttgaggatgatctgaggaggtga

SEQ ID NO: 5 - DNA, 639 bp, Homo sapiens
atggcctccctgttctctggccgcatcctgatccgcaacaatagcgaccaggacgagctggatacggaggctgaggtcagtcgcaggctggagaaccggctggtgctgctgttctttggtgctggggcttgtccacagtgccaggccttcgtgcccatcctcaaggacttcttcgtgcggctcacagatgagttctatgtactgcgggcggctcagctggccctggtgtacgtgtcccaggactccacggaggagcagcaggacctgttcctcaaggacatgccaaagaaatggcttttcctgccctttgaggatgatctgaggagggacctcgggcgccagttctcagtggagcgcctgccggcggtcgtggtgctcaagccggacggggacgtgctcactcgcgacggcgccgacgagatccagcgcctgggcaccgcctgcttcgccaactggcaggaggcggccgaggtgctggaccgcaacttccagctgccagaggacctggaggaccaggagccacggagcctcaccgagtgcctgcgccgccacaagtaccgcgtggaaaaggcggcgcgaggcgggcgcgaccccgggggagggggtggggaggagggcggggccggggggctgttctga

SEQ ID NO: 6 - DNA, 4926 bp, Artificial Sequence
  construct 3
ttggccactccctctctgcgcgctcgctcgctcactgaggccgggcgaccaaaggtcgcccgacgcccgggctttgcccgggcggcctcagtgagcgagcgagcgcgcagagagggagtggccaactccatcactaggggttcctgacattgattattgactagttattaatagtaatcaattacggggtcattagttcatagcccatatatggagttccgcgttacataacttacggtaaatggcccgcctggctgaccgcccaacgacccccgcccattgacgtcaataatgacgtatgttcccatagtaacgccaatagggactttccattgacgtcaatgggtggagtatttacggtaaactgcccacttggcagtacatcaagtgtatcatatgccaagtacgccccctattgacgtcaatgacggtaaatggcccgcctggcattatgcccagtacatgaccttatgggactttcctacttggcagtacatctacgtattagtcatcgctattaccatcgaggtgagccccacgttctgcttcactctccccatctcccccccctccccacccccaattttgtatttatttattttttaattattttgtgcagcgatgggggcggggggggggggggcgcgcgccaggcggggcggggcggggcgaggggcggggcggggcgaggcggagaggtgcggcggcagccaatcagagcggcgcgctccgaaagtttccttttatggcgaggcggcggcggcggcggccctataaaaagcgaagcgcgcggcgggcgggagtcgctgcgttgccttcgccccgtgccccgctccgcgccgcctcgcgccgcccgccccggctctgactgaccgcgttactcccacaggtgagcgggcgggatgagcacggcccggcttcgggtgcggggctccgtgcggggcgtggcgcggggctcgccgtgccgggcggggggtggcggcaggtgggggtgccgggcggggcggggccgcctcgggccggggagggctcgggggaggggcgcggcggccccggagcgccggcggctgtcgaggcgcggcgagccgcagccattgccttttatggtaatcgtgcgagagggcgcagggacttcctttgtcccaaatctggcggagccgaaatctgggaggcgccgccgcaccccctctagcgggcgcgggcgaagcggtgcggcgccggcaggaaggaactgggcggggagggccttcgtgcgtcgccgcgccgccgtccccttctccatctccagcctcggggctgccgcagggggacggctgccttcgggggggacggggcagggcggggttcggcttctggcgtgtgaccggcggcctctgctaaccatgttcatgccttcttctttttcctacagctcctgggcaacgtgctggttattgtgctgtctcatcattttggcaaagaattgccgccaccatggccagcctcttctccggacgcatcctgattcgcaacaattccgaccaagacgaactggataccgaggccgaagtctcgcggagattggagaacaggcttgtgctgctgttctttggcgcgggagcgtgtcctcagtgccaggctttcgtgccaatcctgaaggatttcttcgtgcggctgactgacgaattctacgtcctccgggccgcccagctggcactggtgtacgtgtcccaagactcaaccgaggaacagcaggatctgttcctcaaggacatgcccaaaaagtggctgttcctgccgtttgaggacgacttgcggcgctagaataaaagatctttattttcattagatctgtgtgttggttttttgtgtgatgtcccttatggtgcttctggctctgcagttattagcatagtgttaccatcaaccaccttaacttcatttttcttattcaatacctaggtaggtagatgctagattctggaaataaaatatgagtctcaagtggtccttgtcctctctcccagtcaaattctgaatctagttggcaagattctgaaatcaaggcatataatcagtaataagtgatgatagaagggtatatagaagaattttattatatgagagggtgaaaccctcaaaatgaaatgaaatcagacccttgtcttacaccataaacaaaaataaatttgaatgggttaaagaattaaactaagacctaaaaccataaaaatttttaaagaaatcaaaagaagaaaattctaatattcacgttgcagccgttttttgaatttgatatgagaagcaaaggcaacaaggaggctgaggggtggggaaagggcatgggtgtttcatgaggacagagcttccgtttcatgcaatgaaaagagtttggagacggatggtggtgactggactatacacttacacacggtagcgatggtacactttgtattatgtatattttaccacgatctttttaaagtgtcaaaggcaaatggccaaatggttccttgtcctatagctgtagcagccatcggctgttagtgacaaagcccctgagtcaagatgacagcagcccccataactcctaatcggctctcccgcgtggagtcatttaggagtagtcgcattagagacaagtccaacatctaatcttccaccctggccagggccccagctggcagcgagggtgggagactccgggcagagcagagggcgctgacattggggcccggcctggcttgggtccctctggcctttccccaggggccctctttccttggggctttcttgggccgccactgctcccgctcctctccccccatcccaccccctcaccccctcgttcttcatatccttctctagtgctccctccactttcatccacccttctgcaagagtgtgggaccacaaatgagttttcacctggcctggggacacacgtgcccccacaggtgctgagtgactttctaggacagtaatctgctttaggctaaaatgggacttgatcttctgttagccctaatcatcaattagcagagccggtgaaggtgcagaacctaccgcctttccaggcctcctcccacctctgccacctccactctccttcctgggatgtgggggctggcacacgtgtggcccagggcattggtgggattgcactgagctgggtcattagcgtaatcctggacaagggcagacagggcgagcggagggccagctccggggctcaggcaaggctgggggcttcccccagacaccccactcctcctctgctggacccccacttcatagggcacttcgtgttctcaaagggcttccaaatagcatggtggccttggatgcccagggaagcctcagagttgcttatctccctctagacagaaggggaatctcggtcaagagggagaggtcgccctgttcaaggccacccagccagctcatggcggtaatgggacaaggctggccagccatcccaccctcagaagggacccggtggggcaggtgatctcagaggaggctcacttctgggtctcacattcttggatccggttccaggcctcggccctaaatagtctccctgggctttcaagagaaccacatgagaaaggaggattcgggctctgagcagtttcaccacccaccccccagtctgcaaatcctgacccgtgggtccacctgccccaaaggcggacgcaggacagtagaagggaacagagaacacataaacacagagagggccacagcggctcccacagtcaccgccaccttcctggcggggatgggtggggcgtctgagtttggttcccagcaaatccctctgagccgcccttgcgggctcgcctcaggagcaggggagcaagaggtgggaggaggaggtctaagtcccaggcccaattaagagatcaggtagtgtagggtttgggagcttttaaggtgaagaggcccgggctgatcccacaggccagtataaagcgccgtgaccctcaggtgatgcgccagggccggctgccgtcggggacagggctttccatagccatggcctcactgttctccgggcgcatcctcatccgaaacaacagcgatcaggacgaattggacaccgaggctgaagtctcccgccggctggaaaacaggctcgtgctcctgttcttcggtgccggagcgtgcccgcagtgccaagccttcgtcccaattcttaaggacttctttgtgcgcctcactgatgagttttacgtgctccgggcagcgcagctggccttggtgtatgtgtcgcaagattccactgaggaacaacaggacctgttcctgaaagacatgcctaagaagtggcttttcctgcccttcgaggacgacctgagaagggacctgggacgccagttcagcgtggaacggctgccggccgtcgtggtgctgaagcccgacggggacgtgcttacccgggatggcgctgacgaaatccagaggctgggcaccgcctgtttcgcaaattggcaggaggccgccgaagtgctcgaccggaacttccagctgcccgaggatctggaggaccaggaacctcggtccctgaccgagtgcctcagacgccacaagtaccgcgtggaaaaggccgcgagaggaggacgggacccgggtggcgggggaggcgaagagggcggagccggtggcctgttctgaaacttgtttattgcagcttataatggttacaaataaagcaatagcatcacaaatttcacaaataaagcatttttttcactgcattctagttgtggtttgtccaaactcatcaatgtatcttaaggaacccctagtgatggagttggccactccctctctgcgcgctcgctcgctcactgaggccgggcgaccaaaggtcgcccgacgcccgggctttgcccgggcggcctcagtgagcgagcgagcgcgcagagagggagtggccaa

SEQ ID NO: 7 - DNA, 4942 bp, Artificial Sequence
  construct 6
gcggccgcttggccactccctctctgcgcgctcgctcgctcactgaggccgggcgaccaaaggtcgcccgacgcccgggctttgcccgggcggcctcagtgagcgagcgagcgcgcagagagggagtggccaactccatcactaggggttcctgacattgattattgactagttattaatagtaatcaattacggggtcattagttcatagcccatatatggagttccgcgttacataacttacggtaaatggcccgcctggctgaccgcccaacgacccccgcccattgacgtcaataatgacgtatgttcccatagtaacgccaatagggactttccattgacgtcaatgggtggagtatttacggtaaactgcccacttggcagtacatcaagtgtatcatatgccaagtacgccccctattgacgtcaatgacggtaaatggcccgcctggcattatgcccagtacatgaccttatgggactttcctacttggcagtacatctacgtattagtcatcgctattaccatcgaggtgagccccacgttctgcttcactctccccatctcccccccctccccacccccaattttgtatttatttattttttaattattttgtgcagcgatgggggcggggggggggggggcgcgcgccaggcggggcggggcggggcgaggggcggggcggggcgaggcggagaggtgcggcggcagccaatcagagcggcgcgctccgaaagtttccttttatggcgaggcggcggcggcggcggccctataaaaagcgaagcgcgcggcgggcgggagtcgctgcgttgccttcgccccgtgccccgctccgcgccgcctcgcgccgcccgccccggctctgactgaccgcgttactcccacaggtgagcgggcgggatgagcacggcccggcttcgggtgcggggctccgtgcggggcgtggcgcggggctcgccgtgccgggcggggggtggcggcaggtgggggtgccgggcggggcggggccgcctcgggccggggagggctcgggggaggggcgcggcggccccggagcgccggcggctgtcgaggcgcggcgagccgcagccattgccttttatggtaatcgtgcgagagggcgcagggacttcctttgtcccaaatctggcggagccgaaatctgggaggcgccgccgcaccccctctagcgggcgcgggcgaagcggtgcggcgccggcaggaaggaactgggcggggagggccttcgtgcgtcgccgcgccgccgtccccttctccatctccagcctcggggctgccgcagggggacggctgccttcgggggggacggggcagggcggggttcggcttctggcgtgtgaccggcggcctctgctaaccatgttcatgccttcttctttttcctacagctcctgggcaacgtgctggttattgtgctgtctcatcattttggcaaagaattgccgccaccatggcctccctgttctctggccgcatcctgatccgcaacaatagcgaccaggacgaactggatacggaggctgaggtcagtcgcaggctggagaaccggctggtgctgctgttctttggtgccggggcttgtccacagtgccaggccttcgtgcccatcctcaaggacttcttcgtgcggctcacagatgagttctatgtactgcgggcggctcagctggccctggtgtacgtgtcccaggactccacggaggagcagcaggacctgttcctcaaggacatgccaaagaagtggcttttcctgccctttgaggatgatctgaggaggtagaataaaagatctttattttcattagatctgtgtgttggttttttgtgtgatgtcccttatggtgcttctggctctgcagttattagcatagtgttaccatcaaccaccttaacttcatttttcttattcaatacctaggtaggtagatgctagattctggaaataaaatatgagtctcaagtggtccttgtcctctctcccagtcaaattctgaatctagttggcaagattctgaaatcaaggcatataatcagtaataagtgatgatagaagggtatatagaagaattttattatatgagagggtgaaaccctcaaaatgaaatgaaatcagacccttgtcttacaccataaacaaaaataaatttgaatgggttaaagaattaaactaagacctaaaaccataaaaatttttaaagaaatcaaaagaagaaaattctaatattcacgttgcagccgttttttgaatttgatatgagaagcaaaggcaacaaggaggctgaggggtggggaaagggcatgggtgtttcatgaggacagagcttccgtttcatgcaatgaaaagagtttggagacggatggtggtgactggactatacacttacacacggtagcgatggtacactttgtattatgtatattttaccacgatctttttaaagtgtcaaaggcaaatggccaaatggttccttgtcctatagctgtagcagccatcggctgttagtgacaaagcccctgagtcaagatgacagcagcccccataactcctaatcggctctcccgcgtggagtcatttaggagtagtcgcattagagacaagtccaacatctaatcttccaccctggccagggccccagctggcagcgagggtgggagactccgggcagagcagagggcgctgacattggggcccggcctggcttgggtccctctggcctttccccaggggccctctttccttggggctttcttgggccgccactgctcccgctcctctccccccatcccaccccctcaccccctcgttcttcatatccttctctagtgctccctccactttcatccacccttctgcaagagtgtgggaccacaaatgagttttcacctggcctggggacacacgtgcccccacaggtgctgagtgactttctaggacagtaatctgctttaggctaaaatgggacttgatcttctgttagccctaatcatcaattagcagagccggtgaaggtgcagaacctaccgcctttccaggcctcctcccacctctgccacctccactctccttcctgggatgtgggggctggcacacgtgtggcccagggcattggtgggattgcactgagctgggtcattagcgtaatcctggacaagggcagacagggcgagcggagggccagctccggggctcaggcaaggctgggggcttcccccagacaccccactcctcctctgctggacccccacttcatagggcacttcgtgttctcaaagggcttccaaatagcatggtggccttggatgcccagggaagcctcagagttgcttatctccctctagacagaaggggaatctcggtcaagagggagaggtcgccctgttcaaggccacccagccagctcatggcggtaatgggacaaggctggccagccatcccaccctcagaagggacccggtggggcaggtgatctcagaggaggctcacttctgggtctcacattcttggatccggttccaggcctcggccctaaatagtctccctgggctttcaagagaaccacatgagaaaggaggattcgggctctgagcagtttcaccacccaccccccagtctgcaaatcctgacccgtgggtccacctgccccaaaggcggacgcaggacagtagaagggaacagagaacacataaacacagagagggccacagcggctcccacagtcaccgccaccttcctggcggggatgggtggggcgtctgagtttggttcccagcaaatccctctgagccgcccttgcgggctcgcctcaggagcaggggagcaagaggtgggaggaggaggtctaagtcccaggcccaattaagagatcaggtagtgtagggtttgggagcttttaaggtgaagaggcccgggctgatcccacaggccagtataaagcgccgtgaccctcaggtgatgcgccagggccggctgccgtcggggacagggctttccatagccatggcctccctgttctctggccgcatcctgatccgcaacaatagcgaccaggacgagctggatacggaggctgaggtcagtcgcaggctggagaaccggctggtgctgctgttctttggtgctggggcttgtccacagtgccaggccttcgtgcccatcctcaaggacttcttcgtgcggctcacagatgagttctatgtactgcgggcggctcagctggccctggtgtacgtgtcccaggactccacggaggagcagcaggacctgttcctcaaggacatgccaaagaaatggcttttcctgccctttgaggatgatctgaggagggacctcgggcgccagttctcagtggagcgcctgccggcggtcgtggtgctcaagccggacggggacgtgctcactcgcgacggcgccgacgagatccagcgcctgggcaccgcctgcttcgccaactggcaggaggcggccgaggtgctggaccgcaacttccagctgccagaggacctggaggaccaggagccacggagcctcaccgagtgcctgcgccgccacaagtaccgcgtggaaaaggcggcgcgaggcgggcgcgaccccgggggagggggtggggaggagggcggggccggggggctgttctgaaacttgtttattgcagcttataatggttacaaataaagcaatagcatcacaaatttcacaaataaagcatttttttcactgcattctagttgtggtttgtccaaactcatcaatgtatcttaaggaacccctagtgatggagttggccactccctctctgcgcgctcgctcgctcactgaggccgggcgaccaaaggtcgcccgacgcccgggctttgcccgggcggcctcagtgagcgagcgagcgcgcagagagggagtggccaagcggccgc

SEQ ID NO: 8 - DNA, 4498 bp, Artificial Sequence
  construct 7
gcggccgcttggccactccctctctgcgcgctcgctcgctcactgaggccgggcgaccaaaggtcgcccgacgcccgggctttgcccgggcggcctcagtgagcgagcgagcgcgcagagagggagtggccaactccatcactaggggttcctcacacaaaaaaccaacacacagatctaatgaaaataaagatcttttattctacctcctcagatcatcctcaaagggcaggaaaagccacttctttggcatgtccttgaggaacaggtcctgctgctcctccgtggagtcctgggacacgtacaccagggccagctgagccgcccgcagtacatagaactcatctgtgagccgcacgaagaagtccttgaggatgggcacgaaggcctggcactgtggacaagccccggcaccaaagaacagcagcaccagccggttctccagcctgcgactgacctcagcctccgtatccagttcgtcctggtcgctattgttgcggatcaggatgcggccagagaacagggaggccatggtggcggcaattctttgccaaaatgatgagacagcacaataaccagcacgttgcccaggagctgtaggaaaaagaagaaggcatgaacatggttagcagaggccgccggtcacacgccagaagccgaaccccgccctgccccgtcccccccgaaggcagccgtccccctgcggcagccccgaggctggagatggagaaggggacggcggcgcggcgacgcacgaaggccctccccgcccagttccttcctgccggcgccgcaccgcttcgcccgcgcccgctagagggggtgcggcggcgcctcccagatttcggctccgccagatttgggacaaaggaagtccctgcgccctctcgcacgattaccataaaaggcaatggctgcggctcgccgcgcctcgacagccgccggcgctccggggccgccgcgcccctcccccgagccctccccggcccgaggcggccccgccccgcccggcacccccacctgccgccaccccccgcccggcacggcgagccccgcgccacgccccgcacggagccccgcacccgaagccgggccgtgctcatcccgcccgctcacctgtgggagtaacgcggtcagtcagagccggggcgggcggcgcgaggcggcgcggagcggggcacggggcgaaggcaacgcagcgactcccgcccgccgcgcgcttcgctttttatagggccgccgccgccgccgcctcgccataaaaggaaactttcggagcgcgccgctctgattggctgccgccgcacctctccgcctcgccccgccccgcccctcgccccgccccgccccgcctggcgcgcgccccccccccccccgcccccatcgctgcacaaaataattaaaaaataaataaatacaaaattgggggtggggaggggggggagatggggagagtgaagcagaacgtggggctcacctcgatggtaatagcgatgactaatacgtagatgtactgccaagtaggaaagtcccataaggtcatgtactgggcataatgccaggcgggccatttaccgtcattgacgtcaatagggggcgtacttggcatatgatacacttgatgtactgccaagtgggcagtttaccgtaaatactccacccattgacgtcaatggaaagtccctattggcgttactatgggaacatacgtcattattgacgtcaatgggcgggggtcgttgggcggtcagccaggcgggccatttaccgtaagttatgtaacgcggaactccatatatgggctatgaactaatgaccccgtaattgattactattaataactagtcaataatcaatgtcggaggctgaggggtggggaaagggcatgggtgtttcatgaggacagagcttccgtttcatgcaatgaaaagagtttggagacggatggtggtgactggactatacacttacacacggtagcgatggtacactttgtattatgtatattttaccacgatctttttaaagtgtcaaaggcaaatggccaaatggttccttgtcctatagctgtagcagccatcggctgttagtgacaaagcccctgagtcaagatgacagcagcccccataactcctaatcggctctcccgcgtggagtcatttaggagtagtcgcattagagacaagtccaacatctaatcttccaccctggccagggccccagctggcagcgagggtgggagactccgggcagagcagagggcgctgacattggggcccggcctggcttgggtccctctggcctttccccaggggccctctttccttggggctttcttgggccgccactgctcccgctcctctccccccatcccaccccctcaccccctcgttcttcatatccttctctagtgctccctccactttcatccacccttctgcaagagtgtgggaccacaaatgagttttcacctggcctggggacacacgtgcccccacaggtgctgagtgactttctaggacagtaatctgctttaggctaaaatgggacttgatcttctgttagccctaatcatcaattagcagagccggtgaaggtgcagaacctaccgcctttccaggcctcctcccacctctgccacctccactctccttcctgggatgtgggggctggcacacgtgtggcccagggcattggtgggattgcactgagctgggtcattagcgtaatcctggacaagggcagacagggcgagcggagggccagctccggggctcaggcaaggctgggggcttcccccagacaccccactcctcctctgctggacccccacttcatagggcacttcgtgttctcaaagggcttccaaatagcatggtggccttggatgcccagggaagcctcagagttgcttatctccctctagacagaaggggaatctcggtcaagagggagaggtcgccctgttcaaggccacccagccagctcatggcggtaatgggacaaggctggccagccatcccaccctcagaagggacccggtggggcaggtgatctcagaggaggctcacttctgggtctcacattcttggatccggttccaggcctcggccctaaatagtctccctgggctttcaagagaaccacatgagaaaggaggattcgggctctgagcagtttcaccacccaccccccagtctgcaaatcctgacccgtgggtccacctgccccaaaggcggacgcaggacagtagaagggaacagagaacacataaacacagagagggccacagcggctcccacagtcaccgccaccttcctggcggggatgggtggggcgtctgagtttggttcccagcaaatccctctgagccgcccttgcgggctcgcctcaggagcaggggagcaagaggtgggaggaggaggtctaagtcccaggcccaattaagagatcaggtagtgtagggtttgggagcttttaaggtgaagaggcccgggctgatcccacaggccagtataaagcgccgtgaccctcaggtgatgcgccagggccggctgccgtcggggacagggctttccatagccatggcctccctgttctctggccgcatcctgatccgcaacaatagcgaccaggacgagctggatacggaggctgaggtcagtcgcaggctggagaaccggctggtgctgctgttctttggtgctggggcttgtccacagtgccaggccttcgtgcccatcctcaaggacttcttcgtgcggctcacagatgagttctatgtactgcgggcggctcagctggccctggtgtacgtgtcccaggactccacggaggagcagcaggacctgttcctcaaggacatgccaaagaaatggcttttcctgccctttgaggatgatctgaggagggacctcgggcgccagttctcagtggagcgcctgccggcggtcgtggtgctcaagccggacggggacgtgctcactcgcgacggcgccgacgagatccagcgcctgggcaccgcctgcttcgccaactggcaggaggcggccgaggtgctggaccgcaacttccagctgccagaggacctggaggaccaggagccacggagcctcaccgagtgcctgcgccgccacaagtaccgcgtggaaaaggcggcgcgaggcgggcgcgaccccgggggagggggtggggaggagggcggggccggggggctgttctgaaacttgtttattgcagcttataatggttacaaataaagcaatagcatcacaaatttcacaaataaagcatttttttcactgcattctagttgtggtttgtccaaactcatcaatgtatcttaaggaacccctagtgatggagttggccactccctctctgcgcgctcgctcgctcactgaggccgggcgaccaaaggtcgcccgacgcccgggctttgcccgggcggcctcagtgagcgagcgagcgcgcagagagggagtggccaagcggccgc

SEQ ID NO: 9 - DNA, 5297 bp, Artificial Sequence
  construct 8
gcggccgcttggccactccctctctgcgcgctcgctcgctcactgaggccgggcgaccaaaggtcgcccgacgcccgggctttgcccgggcggcctcagtgagcgagcgagcgcgcagagagggagtggccaactccatcactaggggttcctgacattgattattgactagttattaatagtaatcaattacggggtcattagttcatagcccatatatggagttccgcgttacataacttacggtaaatggcccgcctggctgaccgcccaacgacccccgcccattgacgtcaataatgacgtatgttcccatagtaacgccaatagggactttccattgacgtcaatgggtggagtatttacggtaaactgcccacttggcagtacatcaagtgtatcatatgccaagtacgccccctattgacgtcaatgacggtaaatggcccgcctggcattatgcccagtacatgaccttatgggactttcctacttggcagtacatctacgtattagtcatcgctattaccatcgaggtgagccccacgttctgcttcactctccccatctcccccccctccccacccccaattttgtatttatttattttttaattattttgtgcagcgatgggggcggggggggggggggcgcgcgccaggcggggcggggcggggcgaggggcggggcggggcgaggcggagaggtgcggcggcagccaatcagagcggcgcgctccgaaagtttccttttatggcgaggcggcggcggcggcggccctataaaaagcgaagcgcgcggcgggcgggagtcgctgcgttgccttcgccccgtgccccgctccgcgccgcctcgcgccgcccgccccggctctgactgaccgcgttactcccacaggtgagcgggcgggatgagcacggcccggcttcgggtgcggggctccgtgcggggcgtggcgcggggctcgccgtgccgggcggggggtggcggcaggtgggggtgccgggcggggcggggccgcctcgggccggggagggctcgggggaggggcgcggcggccccggagcgccggcggctgtcgaggcgcggcgagccgcagccattgccttttatggtaatcgtgcgagagggcgcagggacttcctttgtcccaaatctggcggagccgaaatctgggaggcgccgccgcaccccctctagcgggcgcgggcgaagcggtgcggcgccggcaggaaggaactgggcggggagggccttcgtgcgtcgccgcgccgccgtccccttctccatctccagcctcggggctgccgcagggggacggctgccttcgggggggacggggcagggcggggttcggcttctggcgtgtgaccggcggcctctgctaaccatgttcatgccttcttctttttcctacagctcctgggcaacgtgctggttattgtgctgtctcatcattttggcaaagaattgccgccaccatggcctccctgttctctggccgcatcctgatccgcaacaatagcgaccaggacgaactggatacggaggctgaggtcagtcgcaggctggagaaccggctggtgctgctgttctttggtgccggggcttgtccacagtgccaggccttcgtgcccatcctcaaggacttcttcgtgcggctcacagatgagttctatgtactgcgggcggctcagctggccctggtgtacgtgtcccaggactccacggaggagcagcaggacctgttcctcaaggacatgccaaagaagtggcttttcctgccctttgaggatgatctgaggaggtagaataaaagatctttattttcattagatctgtgtgttggttttttgtgtgatgtcccttatggtgcttctggctctgcagttattagcatagtgttaccatcaaccaccttaacttcatttttcttattcaatacctaggtaggtagatgctagattctggaaataaaatatgagtctcaagtggtccttgtcctctctcccagtcaaattctgaatctagttggcaagattctgaaatcaaggcatataatcagtaataagtgatgatagaagggtatatagaagaattttattatatgagagggtgaaaccctcaaaatgaaatgaaatcagacccttgtcttacaccataaacaaaaataaatttgaatgggttaaagaattaaactaagacctaaaaccataaaaatttttaaagaaatcaaaagaagaaaattctaatattcacgttgcagccgttttttgaatttgatatgagaagcaaaggcaacaaaaggacagggaagggagcagtggttcacgcctgtaatcccagcaatttgggaggccaaggtgggtagatcacctgagattaggagttggagaccagcctggccaatatggtgaaaccccgtctctaccaaaaaaacaaaaattagctgagcctggtcatgcatgcctggaatcccaacaactcgggaggctgaggcaggagaatcgcttgaacccaggaggcggagattgcagtgagccaagattgtgccactgcactccagcttggttcccaatagaccccgcaggccctacaggttgtcttcccaacttgccccttgctccataccacccccctccaccccataatattatagaaggacacctagtcagacaaaatgatgcaacttaattttattaggacaaggctggtgggcactggagtggcaacttccagggccaggagaggcactggggaggggtcacagggatgccaccctcagaacagccccccggccccgccctcctccccaccccctcccccggggtcgcgcccgcctcgcgccgccttttccacgcggtacttgtggcggcgcaggcactcggtgaggctccgtggctcctggtcctccaggtcctctggcagctggaagttgcggtccagcacctcggccgcctcctgccagttggcgaagcaggcggtgcccaggcgctggatctcgtcggcgccgtcgcgagtgagcacgtccccgtccggcttgagcaccacgaccgccggcaggcgctccactgagaactggcgcccgaggtccctcctcagatcatcctcaaagggcaggaaaagccatttctttggcatgtccttgaggaacaggtcctgctgctcctccgtggagtcctgggacacgtacaccagggccagctgagccgcccgcagtacatagaactcatctgtgagccgcacgaagaagtccttgaggatgggcacgaaggcctggcactgtggacaagccccagcaccaaagaacagcagcaccagccggttctccagcctgcgactgacctcagcctccgtatccagctcgtcctggtcgctattgttgcggatcaggatgcggccagagaacagggaggccatggctatggaaagccctgtccccgacggcagccggccctggcgcatcacctgagggtcacggcgctttatactggcctgtgggatcagcccgggcctcttcaccttaaaagctcccaaaccctacactacctgatctcttaattgggcctgggacttagacctcctcctcccacctcttgctcccctgctcctgaggcgagcccgcaagggcggctcagagggatttgctgggaaccaaactcagacgccccacccatccccgccaggaaggtggcggtgactgtgggagccgctgtggccctctctgtgtttatgtgttctctgttcccttctactgtcctgcgtccgcctttggggcaggtggacccacgggtcaggatttgcagactggggggtgggtggtgaaactgctcagagcccgaatcctcctttctcatgtggttctcttgaaagcccagggagactatttagggccgaggcctggaaccggatccaagaatgtgagacccagaagtgagcctcctctgagatcacctgccccaccgggtcccttctgagggtgggatggctggccagccttgtcccattaccgccatgagctggctgggtggccttgaacagggcgacctctccctcttgaccgagattccccttctgtctagagggagataagcaactctgaggcttccctgggcatccaaggccaccatgctatttggaagccctttgagaacacgaagtgccctatgaagtgggggtccagcagaggaggagtggggtgtctgggggaagcccccagccttgcctgagccccggagctggccctccgctcgccctgtctgcccttgtccaggattacgctaatgacccagctcagtgcaatcccaccaatgccctgggccacacgtgtgccagcccccacatcccaggaaggagagtggaggtggcagaggtgggaggaggcctggaaaggcggtaggttctgcaccttcaccggctctgctaattgatgattagggctaacagaagatcaagtcccattttagcctaaagcagattactgtcctagaaagtcactcagcacctgtgggggcacgtgtgtccccaggccaggtgaaaactcatttgtggtcccacactcttgcagaagggtggatgaaagtggagggagcactagagaaggatatgaagaacgagggggtgagggggtgggatggggggagaggagcgggagcagtggcggcccaagaaagccccaaggaaagagggcccctggggaaaggccagagggacccaagccaggccgggccccaatgtcagcgccctctgctctgcccggagtctcccaccctcgctgccagctggggccctggccagggtggaagattagatgttggacttgtctctaatgcgactactcctaaatgactccacgcgggagagccgattaggagttatgggggctgctgtcatcttgactcaggggctttgtcactaacagccgatggctgctacagctataggacaaggaaccatttggccatttgcctttgacactttaaaaagatcgtggtaaaatatacataatacaaagtgtaccatcgctaccgtgtgtaagtgtatagtccagtcaccaccatccgtctccaaactcttttcattgcatgaaacggaagctctgtcctcatgaaacacccatgccctttccccacccctcagcctccaggaacccctagtgatggagttggccactccctctctgcgcgctcgctcgctcactgaggccgggcgaccaaaggtcgcccgacgcccgggctttgcccgggcggcctcagtgagcgagcgagcgcgcagagagggagtggccaagcggccgc

SEQ ID NO: 10 - DNA, 4360 bp, Homo sapiens
tcaacaaatgtctcacaattaatacatttggcctaatgttttaggacaagacaaatatttaatttgaacaagagatgtaaaagttaggaattactctagtgaaaacagatttggatgatgatggacaatattagtgtggtgcctcaacaaagacttttgcctcttgcatactattatgattgcacggtaatcttacccagctagtgttttcttaatgtcctggggagcctgatcattgtaaattacctgtgacatctcattaatcctctttttcctcacaaacgcataattaatggtaacattgacaataatacacaaattagctaagtgacgctttatggtgttggttttgattaacgtcaggaacccaaaaatgacgttaatgtaatgcagatcccaaaaggcagtctgcactttgaccccagacatacattttgtttgcaccatcaccaagattaatcctcctctggatgaagatgagacaaaactctggccactggcagtgtgtgctaggctgtcggaaaacaaaccgcctcaactgcatttgtttaagaaggaaatcttaatgcacagaaaacaacggcgtagtgtcatttcctattgtctagttaggacaaagataaatgagcaactgtcatgattcagatcaactgcttccctgctaacttctattatttgcttatttatggactggtgtttaattaaaagtatacctagatatataaaccacatgataaaataattgaaattccttttgctttcactataaatggtttttggaaatcaagactgatttttatatgcatttcaacctgcaggacctttaaatgataaattcttattaaccacaagagggtaaacaaaatcaatgcctgagaaaatatgctttgtctctgacttgagtaacaaagtaaaaacactagaagaaatttggataaagttcttaacttcatcagtgaggcatccttgtagactctgagaaagctgatatagagacgctttttccaaattataaaagagacaaacactttaagtaagtcacagtagcatctactgctgcatcatcaacttctaaattcaggcttaatcatgtgactttaatataaacatgaacagtttcttaattacgattttcacaaatctgagttaagtactgaatctttttaacactccaaagaggtagcatatgctaattttttaaagatgcaaccttctattttcttcgtaacaattacttatagctgaaacatcttaatggtatacattttttaaaaataatagtctcgtatttgattaatttaacatctacttatttaggctatttttcaaaatgttactgctactaaaccacagccctggctaatgatcgtattccacttcaaaaacggagtaagaagaaaagccatattttcatgctttgttctatttttcacacaaataactatcatttatggacaaaaatatgcaacacgtaaagtgatgtcataaaaatttgaaataaatccaccaaaattggaaagcaaagatcaccgaaattatgaaacattgtgggtatatttgataaaaagaagatactatttttgattaaaaaaagagaatatcttaaaaagaagattttggttgctgtgggtatgtattttcaattgtgaggcctctaatccacctctcccccaaaataagaaaacagactgccttacaactgcttgtcatagcagtttaattttgaaaaatgcctcatctgtccctgcttgcaatatattgtcttacgactacgtttaccttttttattttttgggggggggttattgaaagttacaaggagcaaaataatgtttttagagaatttttttcttctcttgtttaaatattattttaaaatcaaaagcagctcatttttaaatcgacatattaagtgttagctgcaccaactttcaccagcacacaaacccattgtaaagcaaactggaatttaaggggcaatggggagtcctacagaggtcatattttcactctgcctaactaaaccataaatcaagattacaacaataaattattttttattattttggcaggaataagtatagccttgaattttgaaagatatttgggcttaattcatatgttaaataggtcgggataaaccaatgctagaagaaattgaaactggcccaatattatacagaaacccaaattaggcactcaccaccaaactaattagtaattgataaatttacaatagtaatgtaatttctttacactgcaaagccaaagaaataggataattgaaagcttcaaatctaaaaaaaaaaaaattgacaatcttttaatcaaaggcattgtttacaacgtggcttttaggtagctgcagtaacatctttaactggttaaaaacactcatcaagctataaaactactttcttagatgtctatagcaaactgtttgaaacctcccaaagtgccttaatttatattttttcagcagctacaatgaatgttactttcttccagtccaaatgtatcattttcacttttcaacttattcaagttcatagagagcaacctatgaagccacaattttatagaaatctatttttcaggtttaaatgtggtaccctgacttttcataagctccaatagttgtgccaagttacttttttgttgttgttctaaggaaagattttatgcaaataaagagactgctctgtgggaaagcatgttttcttaagtatttaatcggacatttccacaccacaacactttgtagacatgtttttgctttgaaaacataatcttatcaggggtggttggtgtacaattcttgtctgttttcttacctttgaatttgagctctatttataaggctcaactaaatgatgtctgcagctaaggcatttccttactagggagttttacacgaacacaattaatatgaaagcacacaacgcattgaacagggtgtcaatttaggtttccggtacaatgtaaccttatcgaagtgttcccgtttacatagaagaaaacaaatatgataaagcggttaaatatgtatctgtcttagatttctaacattttcctctcgatatatcttttcggaataaacaaagggaagtgaattcttcattccttatttgtacaaacaagtgaaattgggtccccttcacgatggaaggcactggcctttctcctcacatggaacaaactgctagagaaacttggtttacacaaaatggaaacatttaatccttgcatctatatttcaaaatagtacatggtttttccataaatctatgtgtgatgacatatttcgtaacattacataaggctttccatgcatttttattcatgggagaatggcttgcagaaaatcacaacattgtactatgcttctccagcaagttaattttcactttactgcgaatatacagtttatggaaaaataatagttatttaagtgtagcgtacttacctgttgctgtgggaaaattcctaccattaaaaatgtgctttcacttcagttattattataatgtaggctataccaatgcctgatgatttttataaacagaacctataaatctgcattttggttcagggctgtactatttagacaaatgaaaatgaagcagcatgacatgaagtccaaaggaacgttcttatacatgcctcaactttggttttttggtaactgccctttggagactatcctttattaaggatcttaatgagggttctgcctgtatttttctcccaagaatgtcaaataaggttcgaaagcaaatgtaaactgtaatacaagtgacacacactaaaaatagccctataaatctgttcattttgtttagatagtctccagagttgtaaaaagtaggactgttcagctttattatttgttttggaaaacctaattctgtagagaataggccactgataatgctatattactttagaggagatttattaagactgtctctagatttaatttttttaaaataaagaaactctttcctgtttttattttccaaataatctacaagataattaactgaatataatctataatattaaataaattttcccatttactcattagaattaagattttgaaaggcacatttatctaaactaaaattaattaaaatttcaaatagaattctcattcctattaacctgtcaaatatgttgcgttcaatgtttccagtaacagaacaacaatatttattatctaacgtaccataagtttttaaaaataactccaggagaacatttttggaacacttacaatctgaatagacaactaaaaaaatcagacatttctgtgtgaaaaatagctattgtaaattaaaatggttgagggagaata

SEQ ID NO: 11 - DNA, 330 bp, Homo sapiens
atggcctccttgttctccggccgaatcctgatccgaaacaatagtgaccaggatgagctggatacagaagctgaggtcagtcgcagactggagaacaggctggtccttctgttctttggtgctggggcttgtcctcagtgccaggccttcgtgcccatcctcaaggacttctttgtgcggctcacggatgagttctatgtactgcgggcagctcaactggctctagtatatgtgtcacaggactccactgaggagcagcaggacctcttcctgaaggacatgccaaagaaatggcttttcctgccctttgaggatgatctgaggaggtag

SEQ ID NO: 12 - DNA, 330 bp, Artificial Sequence
  codon-optimized
atggccagcctcttctccggacgcatcctgattcgcaacaattccgaccaagacgaactggataccgaggccgaagtctcgcggagattggagaacaggcttgtgctgctgttctttggcgcgggagcgtgtcctcagtgccaggctttcgtgccaatcctgaaggatttcttcgtgcggctgactgacgaattctacgtcctccgggccgcccagctggcactggtgtacgtgtcccaagactcaaccgaggaacagcaggatctgttcctcaaggacatgcccaaaaagtggctgttcctgccgtttgaggacgacttgcggcgctag

SEQ ID NO: 13 - DNA, 639 bp, Artificial Sequence
  codon-optimized
atggcctcactgttctccgggcgcatcctcatccgaaacaacagcgatcaggacgaattggacaccgaggctgaagtctcccgccggctggaaaacaggctcgtgctcctgttcttcggtgccggagcgtgcccgcagtgccaagccttcgtcccaattcttaaggacttctttgtgcgcctcactgatgagttttacgtgctccgggcagcgcagctggccttggtgtatgtgtcgcaagattccactgaggaacaacaggacctgttcctgaaagacatgcctaagaagtggcttttcctgcccttcgaggacgacctgagaagggacctgggacgccagttcagcgtggaacggctgccggccgtcgtggtgctgaagcccgacggggacgtgcttacccgggatggcgctgacgaaatccagaggctgggcaccgcctgtttcgcaaattggcaggaggccgccgaagtgctcgaccggaacttccagctgcccgaggatctggaggaccaggaacctcggtccctgaccgagtgcctcagacgccacaagtaccgcgtggaaaaggccgcgagaggaggacgggacccgggtggcgggggaggcgaagagggcggagccggtggcctgttctga

SEQ ID NO: 14 - DNA, 4934 bp, Artificial Sequence
  construct 11
ttggccactccctctctgcgcgctcgctcgctcactgaggccgggcgaccaaaggtcgcccgacgcccgggctttgcccgggcggcctcagtgagcgagcgagcgcgcagagagggagtggccaactccatcactaggggttcctgacattgattattgactagttattaatagtaatcaattacggggtcattagttcatagcccatatatggagttccgcgttacataacttacggtaaatggcccgcctggctgaccgcccaacgacccccgcccattgacgtcaataatgacgtatgttcccatagtaacgccaatagggactttccattgacgtcaatgggtggagtatttacggtaaactgcccacttggcagtacatcaagtgtatcatatgccaagtacgccccctattgacgtcaatgacggtaaatggcccgcctggcattatgcccagtacatgaccttatgggactttcctacttggcagtacatctacgtattagtcatcgctattaccatcgaggtgagccccacgttctgcttcactctccccatctcccccccctccccacccccaattttgtatttatttattttttaattattttgtgcagcgatgggggcggggggggggggggcgcgcgccaggcggggcggggcggggcgaggggcggggcggggcgaggcggagaggtgcggcggcagccaatcagagcggcgcgctccgaaagtttccttttatggcgaggcggcggcggcggcggccctataaaaagcgaagcgcgcggcgggcgggagtcgctgcgttgccttcgccccgtgccccgctccgcgccgcctcgcgccgcccgccccggctctgactgaccgcgttactcccacaggtgagcgggcgggatgagcacggcccggcttcgggtgcggggctccgtgcggggcgtggcgcggggctcgccgtgccgggcggggggtggcggcaggtgggggtgccgggcggggcggggccgcctcgggccggggagggctcgggggaggggcgcggcggccccggagcgccggcggctgtcgaggcgcggcgagccgcagccattgccttttatggtaatcgtgcgagagggcgcagggacttcctttgtcccaaatctggcggagccgaaatctgggaggcgccgccgcaccccctctagcgggcgcgggcgaagcggtgcggcgccggcaggaaggaactgggcggggagggccttcgtgcgtcgccgcgccgccgtccccttctccatctccagcctcggggctgccgcagggggacggctgccttcgggggggacggggcagggcggggttcggcttctggcgtgtgaccggcggcctctgctaaccatgttcatgccttcttctttttcctacagctcctgggcaacgtgctggttattgtgctgtctcatcattttggcaaagaattgccgccaccatggcctccttgttctccggccgaatcctgatccgaaacaatagtgaccaggatgagctggatacagaagctgaggtcagtcgcagactggagaacaggctggtccttctgttctttggtgctggggcttgtcctcagtgccaggccttcgtgcccatcctcaaggacttctttgtgcggctcacggatgagttctatgtactgcgggcagctcaactggctctagtatatgtgtcacaggactccactgaggagcagcaggacctcttcctgaaggacatgccaaagaaatggcttttcctgccctttgaggatgatctgaggaggtagaataaaagatctttattttcattagatctgtgtgttggttttttgtgtgatgtcccttatggtgcttctggctctgcagttattagcatagtgttaccatcaaccaccttaacttcatttttcttattcaatacctaggtaggtagatgctagattctggaaataaaatatgagtctcaagtggtccttgtcctctctcccagtcaaattctgaatctagttggcaagattctgaaatcaaggcatataatcagtaataagtgatgatagaagggtatatagaagaattttattatatgagagggtgaaaccctcaaaatgaaatgaaatcagacccttgtcttacaccataaacaaaaataaatttgaatgggttaaagaattaaactaagacctaaaaccataaaaatttttaaagaaatcaaaagaagaaaattctaatattcacgttgcagccgttttttgaatttgatatgagaagcaaaggcaacaaggaggctgaggggtggggaaagggcatgggtgtttcatgaggacagagcttccgtttcatgcaatgaaaagagtttggagacggatggtggtgactggactatacacttacacacggtagcgatggtacactttgtattatgtatattttaccacgatctttttaaagtgtcaaaggcaaatggccaaatggttccttgtcctatagctgtagcagccatcggctgttagtgacaaagcccctgagtcaagatgacagcagcccccataactcctaatcggctctcccgcgtggagtcatttaggagtagtcgcattagagacaagtccaacatctaatcttccaccctggccagggccccagctggcagcgagggtgggagactccgggcagagcagagggcgctgacattggggcccggcctggcttgggtccctctggcctttccccaggggccctctttccttggggctttcttgggccgccactgctcccgctcctctccccccatcccaccccctcaccccctcgttcttcatatccttctctagtgctccctccactttcatccacccttctgcaagagtgtgggaccacaaatgagttttcacctggcctggggacacacgtgcccccacaggtgctgagtgactttctaggacagtaatctgctttaggctaaaatgggacttgatcttctgttagccctaatcatcaattagcagagccggtgaaggtgcagaacctaccgcctttccaggcctcctcccacctctgccacctccactctccttcctgggatgtgggggctggcacacgtgtggcccagggcattggtgggattgcactgagctgggtcattagcgtaatcctggacaagggcagacagggcgagcggagggccagctccggggctcaggcaaggctgggggcttcccccagacaccccactcctcctctgctggacccccacttcatagggcacttcgtgttctcaaagggcttccaaatagcatggtggccttggatgcccagggaagcctcagagttgcttatctccctctagacagaaggggaatctcggtcaagagggagaggtcgccctgttcaaggccacccagccagctcatggcggtaatgggacaaggctggccagccatcccaccctcagaagggacccggtggggcaggtgatctcagaggaggctcacttctgggtctcacattcttggatccggttccaggcctcggccctaaatagtctccctgggctttcaagagaaccacatgagaaaggaggattcgggctctgagcagtttcaccacccaccccccagtctgcaaatcctgacccgtgggtccacctgccccaaaggcggacgcaggacagtagaagggaacagagaacacataaacacagagagggccacagcggctcccacagtcaccgccaccttcctggcggggatgggtggggcgtctgagtttggttcccagcaaatccctctgagccgcccttgcgggctcgcctcaggagcaggggagcaagaggtgggaggaggaggtctaagtcccaggcccaattaagagatcaggtagtgtagggtttgggagcttttaaggtgaagaggcccgggctgatcccacaggccagtataaagcgccgtgaccctcaggtgatgcgccagggccggctgccgtcggggacagggctttccatagccatggcctccctgttctctggccgcatcctgatccgcaacaatagcgaccaggacgagctggatacggaggctgaggtcagtcgcaggctggagaaccggctggtgctgctgttctttggtgctggggcttgtccacagtgccaggccttcgtgcccatcctcaaggacttcttcgtgcggctcacagatgagttctatgtactgcgggcggctcagctggccctggtgtacgtgtcccaggactccacggaggagcagcaggacctgttcctcaaggacatgccaaagaaatggcttttcctgccctttgaggatgatctgaggagggacctcgggcgccagttctcagtggagcgcctgccggcggtcgtggtgctcaagccggacggggacgtgctcactcgcgacggcgccgacgagatccagcgcctgggcaccgcctgcttcgccaactggcaggaggcggccgaggtgctggaccgcaacttccagctgccagaggacctggaggaccaggagccacggagcctcaccgagtgcctgcgccgccacaagtaccgcgtggaaaaggcggcgcgaggcgggcgcgaccccgggggagggggtggggaggagggcggggccggggggctgttctgaaacttgtttattgcagcttataatggttacaaataaagcaatagcatcacaaatttcacaaataaagcatttttttcactgcattctagttgtggtttgtccaaactcatcaatgtatcttaaggaacccctagtgatggagttggccactccctctctgcgcgctcgctcgctcactgaggccgggcgaccaaaggtcgcccgacgcccgggctttgcccgggcggcctcagtgagcgagcgagcgcgcagagagggagtggccaagcggccgc

SEQ ID NO: 15 - DNA, 12646 bp, artificial sequence
  CT35
tagaaaaactcatcgagcatcaaatgaaattgcaatttattcatatcaggattatcaataccatatttttgaaaaagccgtttctgtaatgaaggagaaaactcaccgaggcagttccataggatggcaagatcctggtatcggtctgcgattccgactcgtccaacatcaatacaacctattaatttcccctcgtcaaaaataaggttatcaagtgagaaatcaccatgagtgacgactgaatccggtgagaatggcaaaagtttatgcatttctttccagacttgttcaacaggccagccattacgctcgtcatcaaaatcactcgcatcaaccaaaccgttattcattcgtgattgcgcctgagcgaggcgaaatacgcgatcgctgttaaaaggacaattacaaacaggaatcgagtgcaaccggcgcaggaacactgccagcgcatcaacaatattttcacctgaatcaggatattcttctaatacctggaacgctgtttttccggggatcgcagtggtgagtaaccatgcatcatcaggagtacggataaaatgcttgatggtcggaagtggcataaattccgtcagccagtttagtctgaccatctcatctgtaacatcattggcaacgctacctttgccatgtttcagaaacaactctggcgcatcgggcttcccatacaagcgatagattgtcgcacctgattgcccgacattatcgcgagcccatttatacccatataaatcagcatccatgttggaatttaatcgcggcctcgacgtttcccgttgaatatggctcatattcttcctttttcaatattattgaagcatttatcagggttattgtctcatgagcggatacatatttgaatgtatttagaaaaataaacaaataggggtcagtgttacaaccaattaaccaattctgaacattatcgcgagcccatttatacctgaatatggctcataacaccccttgtttgcctggcggcagtagcgcggtggtcccacctgaccccatgccgaactcagaagtgaaacgccgtagcgccgatggtagtgtggggactccccatgcgagagtagggaactgccaggcatcaaataaaacgaaaggctcagtcgaaagactgggcctttcgcccgggctaattagggggtgtcgcccttattcgactctatagtgaagttcctattctctagaaagtataggaacttctgaagtggggtcgacttaattaaggctgcgcgctcgctcgctcactgaggccgcccgggcaaagcccgggcgtcgggcgacctttggtcgcccggcctcagtgagcgagcgagcgcgcagagagggagtggccaactccatcactaggggttccttgtagttaatgattaacccgccatgctacttatctacgtagcaagctagctagttattaatagtaatcaattacggggtcattagttcatagcccatatatggagttccgcgttacataacttacggtaaatggcccgcctggctgaccgcccaacgacccccgcccattgacgtcaataatgacgtatgttcccatagtaacgccaatagggactttccattgacgtcaatgggtggagtatttacggtaaactgcccacttggcagtacatcaagtgtatcatatgccaagtacgccccctattgacgtcaatgacggtaaatggcccgcctggcattatgcccagtacatgaccttatgggactttcctacttggcagtacatctacgtattagtcatcgctattaacatggtcgaggtgagccccacgttctgcttcactctccccatctcccccccctccccacccccaattttgtatttatttattttttaattattttgtgcagcgatgggggcggggggggggggggggcgcgcgccaggcggggcggggcggggcgaggggcggggcggggcgaggcggagaggtgcggcggcagccaatcagagcggcgcgctccgaaagtttccttttatggcgaggcggcggcggcggcggccctataaaaagcgaagcgcgcggcgggcgggagtcgctgcgcgctgccttcgccccgtgccccgctccgccgccgcctcgcgccgcccgccccggctctgactgaccgcgttactcccacaggtgagcgggcgggagcacggcccggcttcgggtgcggggctccgtacggggcgtggcgcggggctcgccgtgccgggcggggggtggcggcaggtgggggtgccgggcggggcggggccgcctcgggccggggagggctcgggggaggggcgcggcggcccccggagcgccggcggctgtcgaggcgcggcgagccgcagccattgccttttatggtaatcgtgcgagagggcgcagggacttcctttgtcccaaatctgtgcggagccgaaatctgggaggcgccgccgcaccccctctagcgggcgcggggcgaagcggtgcggcgccggcaggaaggaaatgggcggggagggccttcgtgcgtcgccgcgccgccgtccccttctccctctccagcctcggggctgtccgcggggggacggctgccttcgggggggacggggcagggcggggttcggcttctggcgtgtgaccggcggctctagacaattgtactaaccttcttctctttcctctcctgacaggttggtgtacactagcggccgccaccatggccagcctcttctccggacgcatcctgattcgcaacaattccgaccaagacgaactggataccgaggccgaagtctcgcggagattggagaacaggcttgtgctgctgttctttggcgcgggagcgtgtcctcagtgccaggctttcgtgccaatcctgaaggatttcttcgtgcggctgactgacgaattctacgtcctccgggccgcccagctggcactggtgtacgtgtcccaagactcaaccgaggaacagcaggatctgttcctcaaggacatgcccaaaaagtggctgttcctgccgtttgaggacgacttgcggcgctagtgatcagcctcgactgtgccttctagttgccagccatctgttgtttgcccctcccccgtgccttccttgaccctggaaggtgccactcccactgtcctttcctaataaaatgaggaaattgcatcgcattgtctgagtaggtgtcattctattctggggggtggggtggggcaggacagcaagggggaggattgggaagacaatagcaggcatgctggggaggatccaatttattctaaatgcataataaatactgataacatcttatagtttgtattatattttgtattatcgttgacatgtataattttgatatcaaaaactgattttccctttattattttcgagatttattttcttaattctctttaacaaactagaaatattgtatatacaaaaaatcataaataatagatgaatagtttaattataggtgttcatcaatcgaaaaagcaacgtatcttatttaaagtgcgttgcttttttctcatttataaggttaaataattctcatatatcaagcaaagtgacaggcgcccttaaatattctgacaaatgctctttccctaaactccccccataaaaaaacccgccgaagcgggtttttacgttatttgcggattaacgattactcgttatcagaaccgcccaggaagctttagttattaatagtaatcaattacggggtcattagttcatagcccatatatggagttccgcgttacataacttacggtaaatggcccgcctggctgaccgcccaacgacccccgcccattgacgtcaataatgacgtatgttcccatagtaacgccaatagggactttccattgacgtcaatgggtggagtatttacggtaaactgcccacttggcagtacatcaagtgtatcatatgccaagtacgccccctattgacgtcaatgacggtaaatggcccgcctggcattatgcccagtacatgaccttatgggactttcctacttggcagtacatctacgtattagtcatcgctattaacatggtcgaggtgagccccacgttctgcttcactctccccatctcccccccctccccacccccaattttgtatttatttattttttaattattttgtgcagcgatgggggcggggggggggggggggcgcgcgccaggcggggcggggcggggcgaggggcggggcggggcgaggcggagaggtgcggcggcagccaatcagagcggcgcgctccgaaagtttccttttatggcgaggcggcggcggcggcggccctataaaaagcgaagcgcgcggcgggcggggagtcgctgcgacgctgccttcgccccgtgccccgctccgccgccgcctcgcgccgcccgccccggctctgactgaccgcgttactcccacaggtgagcgggcgggatgagcacggcccggcttcgggtgcggggctccgtacggggcgtggcgcggggctcgccgtgccgggcggggggtggcggcaggtgggggtgccgggcggggcggggccgcctcgggccggggagggctcgggggaggggcgcggcggcccccggagcgccggcggctgtcgaggcgcggcgagccgcagccattgccttttatggtaatcgtgcgagagggcgcagggacttcctttgtcccaaatctgtgcggagccgaaatctgggaggcgccgccgcaccccctctagcgggcgcggggcgaagcggtgcggcgccggcaggaaggaaatgggcggggagggccttcgtgcgtcgccgcgccgccgtccccttctccctctccagcctcggggctgtccgcggggggacggctgccttcgggggggacggggcagggcggggttcggcttctggcgtgtgaccggcggctctagacaattgtactaaccttcttctctttcctctcctgacaggttggtgtacactaggccatacaggccgccaccatggcctcactgttctccgggcgcatcctcatccgaaacaacagcgatcaggacgaattggacaccgaggctgaagtctcccgccggctggaaaacaggctcgtgctcctgttcttcggtgccggagcgtgcccgcagtgccaagccttcgtcccaattcttaaggacttctttgtgcgcctcactgatgagttttacgtgctccgggcagcgcagctggccttggtgtatgtgtcgcaagattccactgaggaacaacaggacctgttcctgaaagacatgcctaagaagtggcttttcctgcccttcgaggacgacctgagaagggacctgggacgccagttcagcgtggaacggctgccggccgtcgtggtgctgaagcccgacggggacgtgcttacccgggatggcgctgacgaaatccagaggctgggcaccgcctgtttcgcaaattggcaggaggccgccgaagtgctcgaccggaacttccagctgcccgaggatctggaggaccaggaacctcggtccctgaccgagtgcctcagacgccacaagtaccgcgtggaaaaggccgcgagaggaggacgggacccgggtggcgggggaggcgaagagggcggagccggtggcctgttctgatagatctgcctcgactgtgccttctagttgccagccatctgttgtttgcccctcccccgtgccttccttgaccctggaaggtgccactcccactgtcctttcctaataaaatgaggaaattgcatcgcattgtctgagtaggtgtcattctattctggggggtggggtggggcaggacagcaagggggaggattgggaagacaatagcaggcatgctggggactcgagttctacgtagataagtagcatggcgggttaatcattaactacaaggaacccctagtgatggagttggccactccctctctgcgcgctcgctcgctcactgaggccgggcgaccaaaggtcgcccgacgcccgggctttgcccgggcggcctcagtgagcgagcgagcgcgcagccttaattaacctaaggaaaatgaagtgaagttcctatactttctagagaataggaacttctatagtgagtcgaataagggcgacacaaaatttattctaaatgcataataaatactgataacatcttatagtttgtattatattttgtattatcgttgacatgtataattttgatatcaaaaactgattttccctttattattttcgagatttattttcttaattctctttaacaaactagaaatattgtatatacaaaaaatcataaataatagatgaatagtttaattataggtgttcatcaatcgaaaaagcaacgtatcttatttaaagtgcgttgcttttttctcatttataaggttaaataattctcatatatcaagcaaagtgacaggcgcccttaaatattctgacaaatgctctttccctaaactccccccataaaaaaacccgccgaagcgggtttttacgttatttgcggattaacgattactcgttatcagaaccgcccagggggcccgagcttaacctttttatttgggggagagggaagtcatgaaaaaactaacctttgaaattcgatctccagcacatcagcaaaacgctattcacgcagtacagcaaatccttccagacccaaccaaaccaatcgtagtaaccattcaggaacgcaaccgcagcttagaccaaaacaggaagctatgggcctgcttaggtgacgtctctcgtcaggttgaatggcatggtcgctggctggatgcagaaagctggaagtgtgtgtttaccgcagcattaaagcagcaggatgttgttcctaaccttgccgggaatggctttgtggtaataggccagtcaaccagcaggatgcgtgtaggcgaatttgcggagctattagagcttatacaggcattcggtacagagcgtggcgttaagtggtcagacgaagcgagactggctctggagtggaaagcgagatggggagacagggctgcatgataaatgtcgttagtttctccggtggcaggacgtcagcatatttgctctggctaatggagcaaaagcgacgggcaggtaaagacgtgcattacgttttcatggatacaggttgtgaacatccaatgacatatcggtttgtcagggaagttgtgaagttctgggatataccgctcaccgtattgcaggttgatatcaacccggagcttggacagccaaatggttatacggtatgggaaccaaaggatattcagacgcgaatgcctgttctgaagccatttatcgatatggtaaagaaatatggcactccatacgtcggcggcgcgttctgcactgacagattaaaactcgttcccttcaccaaatactgtgatgaccatttcgggcgagggaattacaccacgtggattggcatcagagctgatgaaccgaagcggctaaagccaaagcctggaatcagatatcttgctgaactgtcagactttgagaaggaagatatcctcgcatggtggaagcaacaaccattcgatttgcaaataccggaacatctcggtaactgcatattctgcattaaaaaatcaacgcaaaaaatcggacttgcctgcaaagatgaggagggattgcagcgtgtttttaatgaggtcatcacgggatcccatgtgcgtgacggacatcgggaaacgccaaaggagattatgtaccgaggaagaatgtcgctggacggtatcgcgaaaatgtattcagaaaatgattatcaagccctgtatcaggacatggtacgagctaaaagattcgataccggctcttgttctgagtcatgcgaaatatttggagggcagcttgatttcgacttcgggagggaagctgcatgatgcgatgttatcggtgcggtgaatgcaaagaagataaccgcttccgaccaaatcaaccttactggaatcgatggtgtctccggtgtgaaagaacaccaacaggggtgttaccactaccgcaggaaaaggaggacgtgtggcgagacagcgacgaagtatcaccgacataatctgcgaaaactgcaaataccttccaacgaaacgcaccagaaataaacccaagccaatcccaaaagaatctgacgtaaaaaccttcaactacacggctcacctgtgggatatccggtggctaagacgtcgtgcgaggaaaacaaggtgattgaccaaaatcgaagttacgaacaagaaagcgtcgagcgagctttaacgtgcgctaactgcggtcagaagctgcatgtgctggaagttcacgtgtgtgagcactgctgcgcagaactgatgagcgatccgaatagctcgatgcacgaggaagaagatgatggctaaaccagcgcgaagacgatgtaaaaacgatgaatgccgggaatggtttcaccctgcattcgctaatcagtggtggtgctctccagagtgtggaaccaagatagcactcgaacgacgaagtaaagaacgcgaaaaagcggaaaaagcagcagagaagaaacgacgacgagaggagcagaaacagaaagataaacttaagattcgaaaactcgccttaaagccccgcagttactggattaaacaagcccaacaagccgtaaacgccttcatcagagaaagagaccgcgacttaccatgtatctcgtgcggaacgctcacgtctgctcagtgggatgccggacattaccggacaactgctgcggcacctcaactccgatttaatgaacgcaatattcacaagcaatgcgtggtgtgcaaccagcacaaaagcggaaatctcgttccgtatcgcgtcgaactgattagccgcatcgggcaggaagcagtagacgaaatcgaatcaaaccataaccgccatcgctggactatcgaagagtgcaaggcgatcaaggcagagtaccaacagaaactcaaagacctgcgaaatagcagaagtgaggccgcatgacgttctcagtaaaaaccattccagacatgctcgttgaaacatacggaaatcagacagaagtagcacgcagactgaaatgtagtcgcggtacggtcagaaaatacgttgatgataaagacgggaaaatgcacgccatcgtcaacgacgttctcatggttcatcgcggatggagtgaaagagatgcgctattacgaaaaaattgatggcagcaaataccgaaatatttgggtagttggcgatctgcacggatgctacacgaacctgatgaacaaactggatacgattggattcgacaacaaaaaagacctgcttatctcggtgggcgatttggttgatcgtggtgcagagaacgttgaatgcctggaattaatcacattcccctggttcagagctgtacgtggaaaccatgagcaaatgatgattgatggcttatcagagcgtggaaacgttaatcactggctgcttaatggcggtggctggttctttaatctcgattacgacaaagaaattctggctaaagctcttgcccataaagcagatgaacttccgttaatcatcgaactggtgagcaaagataaaaaatatgttatctgccacgccgattatccctttgacgaatacgagtttggaaagccagttgatcatcagcaggtaatctggaaccgcgaacgaatcagcaactcacaaaacgggatcgtgaaagaaatcaaaggcgcggacacgttcatctttggtcatacgccagcagtgaaaccactcaagtttgccaaccaaatgtatatcgataccggcgcagtgttctgcggaaacctaacattgattcaggtacagggagaaggcgcatgagactcgaaagcgtagctaaatttcattcgccaaaaagcccgatgatgagcgactcaccacgggccacggcttctgactctctttccggtactgatgtgatggctgctatggggatggcgcaatcacaagccggattcggtatggctgcattctgcggtaagcacgaactcagccagaacgacaaacaaaaggctatcaactatctgatgcaatttgcacacaaggtatcggggaaataccgtggtgtggcaaagcttgaaggaaatactaaggcaaaggtactgcaagtgctcgcaacattcgcttatgcggattattgccgtagtgccgcgacgccgggggcaagatgcagagattgccatggtacaggccgtgcggttgatattgccaaaacagagctgtgggggagagttgtcgagaaagagtgcggaagatgcaaaggcgtcggctattcaaggatgccagcaagcgcagcatatcgcgctgtgacgatgctaatcccaaaccttacccaacccacctggtcacgcactgttaagccgctgtatgacgctctggtggtgcaatgccacaaagaagagtcaatcgcagacaacattttgaatgcggtcacacgttagcagcatgattgccacggatggcaacatattaacggcatgatattgacttattgaataaaattgggtaaatttgactcaacgatgggttaattcgctcgttgtggtagtgagatgaaaagaggcggcgcttactaccgattccgcctagttggtcacttcgacgtatcgtctggaactccaaccatcgcaggcagagaggtctgcaaaatgcaatcccgaaacagttcgcaggtaatagttagagcctgcataacggtttcgggattttttatatctgcacaacaggtaagagcattgagtcgataatcgtgaagagtcggcgagcctggttagccagtgctctttccgttgtgctgaattaagcgaataccggaagcagaaccggatcaccaaatgcgtacaggcgtcatcgccgcccagcaacagcacaacccaaactgagccgtagccactgtctgtcctgaattcattagtaatagttacgctgcggccttttacacatgaccttcgtgaaagcgggtggcaggaggtcgcgctaacaacctcctgccgttttgcccgtgcatatcggtcacgaacaaatctgattactaaacacagtagcctggatttgttctatcagtaatcgaccttattcctaattaaatagagcaaatccccttattgggggtaagacatgaagatgccagaaaaacatgacctgttggccgccattctcgcggcaaaggaacaaggcatcggggcaatccttgcgtttgcaatggcgtaccttcgcggcagatataatggcggtgcgtttacaaaaacagtaatcgacgcaacgatgtgcgccattatcgcctagttcattcgtgaccttctcgacttcgccggactaagtagcaatctcgcttatataacgagcgtgtttatcggctacatcggtactgactcgattggttcgcttatcaaacgcttcgctgctaaaaaagccggagtagaagatggtagaaatcaataatcaacgtaaggcgttcctcgatatgctggcgtggtcggagggaactgataacggacgtcagaaaaccagaaatcatggttatgacgtcattgtaggcggagagctatttactgattactccgatcaccctcgcaaacttgtcacgctaaacccaaaactcaaatcaacaggctaagactggccgtcgttttacaacacagaaagagtttgtagaaacgcaaaaaggccatccgtcaggggccttctgcttagtttgatgcctggcagttccctactctcgccttccgcttcctcgctcactgactcgctgcgctcggtcgttcggctgcggcgagcggtatcagctcactcaaaggcggtaatacggttatccacagaatcaggggataacgcaggaaagaacatgtgagcaaaaggccagcaaaaggccaggaaccgtaaaaaggccgcgttgctggcgtttttccataggctccgcccccctgacgagcatcacaaaaatcgacgctcaagtcagaggtggcgaaacccgacaggactataaagataccaggcgtttccccctggaagctccctcgtgcgctctcctgttccgaccctgccgcttaccggatacctgtccgcctttctcccttcgggaagcgtggcgctttctcatagctcacgctgtaggtatctcagttcggtgtaggtcgttcgctccaagctgggctgtgtgcacgaaccccccgttcagcccgaccgctgcgccttatccggtaactatcgtcttgagtccaacccggtaagacacgacttatcgccactggcagcagccactggtaacaggattagcagagcgaggtatgtaggcggtgctacagagttcttgaagtggtgggctaactacggctacactagaagaacagtatttggtatctgcgctctgctgaagccagttaccttcggaaaaagagttggtagctcttgatccggcaaacaaaccaccgctggtagcggtggtttttttgtttgcaagcagcagattacgcgcagaaaaaaaggatctcaagaagatcctttgatcttttctacggggtctgacgctcagtggaacgacgcgcgcgtaactcacgttaagggattttggtcatgagcttgcgccgtcccgtcaagtcagcgtaatgctctgct

SEQ ID NO: 16 - DNA, 12451 bp, artificial sequence
  CT37
tagaaaaactcatcgagcatcaaatgaaattgcaatttattcatatcaggattatcaataccatatttttgaaaaagccgtttctgtaatgaaggagaaaactcaccgaggcagttccataggatggcaagatcctggtatcggtctgcgattccgactcgtccaacatcaatacaacctattaatttcccctcgtcaaaaataaggttatcaagtgagaaatcaccatgagtgacgactgaatccggtgagaatggcaaaagtttatgcatttctttccagacttgttcaacaggccagccattacgctcgtcatcaaaatcactcgcatcaaccaaaccgttattcattcgtgattgcgcctgagcgaggcgaaatacgcgatcgctgttaaaaggacaattacaaacaggaatcgagtgcaaccggcgcaggaacactgccagcgcatcaacaatattttcacctgaatcaggatattcttctaatacctggaacgctgtttttccggggatcgcagtggtgagtaaccatgcatcatcaggagtacggataaaatgcttgatggtcggaagtggcataaattccgtcagccagtttagtctgaccatctcatctgtaacatcattggcaacgctacctttgccatgtttcagaaacaactctggcgcatcgggcttcccatacaagcgatagattgtcgcacctgattgcccgacattatcgcgagcccatttatacccatataaatcagcatccatgttggaatttaatcgcggcctcgacgtttcccgttgaatatggctcatattcttcctttttcaatattattgaagcatttatcagggttattgtctcatgagcggatacatatttgaatgtatttagaaaaataaacaaataggggtcagtgttacaaccaattaaccaattctgaacattatcgcgagcccatttatacctgaatatggctcataacaccccttgtttgcctggcggcagtagcgcggtggtcccacctgaccccatgccgaactcagaagtgaaacgccgtagcgccgatggtagtgtggggactccccatgcgagagtagggaactgccaggcatcaaataaaacgaaaggctcagtcgaaagactgggcctttcgcccgggctaattagggggtgtcgcccttattcgactctatagtgaagttcctattctctagaaagtataggaacttctgaagtggggtcgacttaattaaggctgcgcgctcgctcgctcactgaggccgcccgggcaaagcccgggcgtcgggcgacctttggtcgcccggcctcagtgagcgagcgagcgcgcagagagggagtggccaactccatcactaggggttccttgtagttaatgattaacccgccatgctacttatctacgtagcaagctagctagttattaatagtaatcaattacggggtcattagttcatagcccatatatggagttccgcgttacataacttacggtaaatggcccgcctggctgaccgcccaacgacccccgcccattgacgtcaataatgacgtatgttcccatagtaacgccaatagggactttccattgacgtcaatgggtggagtatttacggtaaactgcccacttggcagtacatcaagtgtatcatatgccaagtacgccccctattgacgtcaatgacggtaaatggcccgcctggcattatgcccagtacatgaccttatgggactttcctacttggcagtacatctacgtattagtcatcgctattaacatggtcgaggtgagccccacgttctgcttcactctccccatctcccccccctccccacccccaattttgtatttatttattttttaattattttgtgcagcgatgggggcggggggggggggggggcgcgcgccaggcggggcggggcggggcgaggggcggggcggggcgaggcggagaggtgcggcggcagccaatcagagcggcgcgctccgaaagtttccttttatggcgaggcggcggcggcggcggccctataaaaagcgaagcgcgcggcgggcgggagtcgctgcgcgctgccttcgccccgtgccccgctccgccgccgcctcgcgccgcccgccccggctctgactgaccgcgttactcccacaggtgagcgggcgggagcacggcccggcttcgggtgcggggctccgtacggggcgtggcgcggggctcgccgtgccgggcggggggtggcggcaggtgggggtgccgggcggggcggggccgcctcgggccggggagggctcgggggaggggcgcggcggcccccggagcgccggcggctgtcgaggcgcggcgagccgcagccattgccttttatggtaatcgtgcgagagggcgcagggacttcctttgtcccaaatctgtgcggagccgaaatctgggaggcgccgccgcaccccctctagcgggcgcggggcgaagcggtgcggcgccggcaggaaggaaatgggcggggagggccttcgtgcgtcgccgcgccgccgtccccttctccctctccagcctcggggctgtccgcggggggacggctgccttcgggggggacggggcagggcggggttcggcttctggcgtgtgaccggcggctctagacaattgtactaaccttcttctctttcctctcctgacaggttggtgtacactagcggccgccaccatggcctccctgttctctggccgcatcctgatccgcaacaatagcgaccaggacgagctggatacggaggctgaggtcagtcgcaggctggagaaccggctggtgctgctgttctttggtgctggggcttgtccacagtgccaggccttcgtgcccatcctcaaggacttcttcgtgcggctcacagatgagttctatgtactgcgggcggctcagctggccctggtgtacgtgtcccaggactccacggaggagcagcaggacctgttcctcaaggacatgccaaagaaatggcttttcctgccctttgaggatgatctgaggaggtgatcatctcatggatccaagagatctgcctcgactgtgccttctagttgccagccatctgttgtttgcccctcccccgtgccttccttgaccctggaaggtgccactcccactgtcctttcctaataaaatgaggaaattgcatcgcattgtctgagtaggtgtcattctattctggggggtggggtggggcaggacagcaagggggaggattgggaagacaatagcaggcatgctggggactcgaaaggaaaatgaagtgaagttcctatactttctagagaataggaacttctatagtgagtcgaataagggcgacacaaaatttattctaaatgcataataaatactgataacatcttatagtttgtattatattttgtattatcgttgacatgtataattttgatatcaaaaactgattttccctttattattttcgagatttattttcttaattctctttaacaaactagaaatattgtatatacaaaaaatcataaataatagatgaatagtttaattataggtgttcatcaatcgaaaaagcaacgtatcttatttaaagtgcgttgcttttttctcatttataaggttaaataattctcatatatcaagcaaagtgacaggcgcccttaaatattctgacaaatgctctttccctaaactccccccataaaaaaacccgccgaagcgggtttttacgttatttgcggattaacgattactcgttatcagaaccgcccagggggcccgagcttactagctagttattaatagtaatcaattacggggtcattagttcatagcccatatatggagttccgcgttacataacttacggtaaatggcccgcctggctgaccgcccaacgacccccgcccattgacgtcaataatgacgtatgttcccatagtaacgccaatagggactttccattgacgtcaatgggtggagtatttacggtaaactgcccacttggcagtacatcaagtgtatcatatgccaagtacgccccctattgacgtcaatgacggtaaatggcccgcctggcattatgcccagtacatgaccttatgggactttcctacttggcagtacatctacgtattagtcatcgctattaacatggtcgaggtgagccccacgttctgcttcactctccccatctcccccccctccccacccccaattttgtatttatttattttttaattattttgtgcagcgatgggggcggggggggggggggggcgcgcgccaggcggggcggggcggggcgaggggcggggcggggcgaggcggagaggtgcggcggcagccaatcagagcggcgcgctccgaaagtttccttttatggcgaggcggcggcggcggcggccctataaaaagcgaagcgcgcggcgggcggggagtcgctgcgcgctgccttcgccccgtgccccgctccgccgccgcctcgcgccgcccgccccggctctgactgaccgcgttactcccacaggtgagcgggcgggatgagcacggcccggcttcgggtgcggggctccgtacggggcgtggcgcggggctcgccgtgccgggcggggggtggcggcaggtgggggtgccgggcggggcggggccgcctcgggccggggagggctcgggggaggggcgcggcggcccccggagcgccggcggctgtcgaggcgcggcgagccgcagccattgccttttatggtaatcgtgcgagagggcgcagggacttcctttgtcccaaatctgtgcggagccgaaatctgggaggcgccgccgcaccccctctagcgggcgcggggcgaagcggtgcggcgccggcaggaaggaaatgggcggggagggccttcgtgcgtcgccgcgccgccgtccccttctccctctccagcctcggggctgtccgcggggggacggctgccttcgggggggacggggcagggcggggttcggcttctggcgtgtgaccggcggctctagacaattgtactaaccttcttctctttcctctcctgacaggttggtgtacactagcggccgccaccatggcctccctgttctctggccgcatcctgatccgcaacaatagcgaccaggacgagctggatacggaggctgaggtcagtcgcaggctggagaaccggctggtgctgctgttctttggtgctggggcttgtccacagtgccaggccttcgtgcccatcctcaaggacttcttcgtgcggctcacagatgagttctatgtactgcgggcggctcagctggccctggtgtacgtgtcccaggactccacggaggagcagcaggacctgttcctcaaggacatgccaaagaaatggcttttcctgccctttgaggatgatctgaggaggtgatcatctcatggatccaagagatctgcctcgactgtgccttctagttgccagccatctgttgtttgcccctcccccgtgccttccttgaccctggaaggtgccactcccactgtcctttcctaataaaatgaggaaattgcatcgcattgtctgagtaggtgtcattctattctggggggtggggtggggcaggacagcaagggggaggattgggaagacaatagcaggcatgctggggactcgagttctacgtagataagtagcatggcgggttaatcattaactacaaggaacccctagtgatggagttggccactccctctctgcgcgctcgctcgctcactgaggccgggcgaccaaaggtcgcccgacgcccgggctttgcccgggcggcctcagtgagcgagcgagcgcgcagccttaattaacctaaggaaaatgaagtgaagttcctatactttctagagaataggaacttctatagtgagtcgaataagggcgacacaaaatttattctaaatgcataataaatactgataacatcttatagtttgtattatattttgtattatcgttgacatgtataattttgatatcaaaaactgattttccctttattattttcgagatttattttcttaattctctttaacaaactagaaatattgtatatacaaaaaatcataaataatagatgaatagtttaattataggtgttcatcaatcgaaaaagcaacgtatcttatttaaagtgcgttgcttttttctcatttataaggttaaataattctcatatatcaagcaaagtgacaggcgcccttaaatattctgacaaatgctctttccctaaactccccccataaaaaaacccgccgaagcgggtttttacgttatttgcggattaacgattactcgttatcagaaccgcccagggggcccgagcttaacctttttatttgggggagagggaagtcatgaaaaaactaacctttgaaattcgatctccagcacatcagcaaaacgctattcacgcagtacagcaaatccttccagacccaaccaaaccaatcgtagtaaccattcaggaacgcaaccgcagcttagaccaaaacaggaagctatgggcctgcttaggtgacgtctctcgtcaggttgaatggcatggtcgctggctggatgcagaaagctggaagtgtgtgtttaccgcagcattaaagcagcaggatgttgttcctaaccttgccgggaatggctttgtggtaataggccagtcaaccagcaggatgcgtgtaggcgaatttgcggagctattagagcttatacaggcattcggtacagagcgtggcgttaagtggtcagacgaagcgagactggctctggagtggaaagcgagatggggagacagggctgcatgataaatgtcgttagtttctccggtggcaggacgtcagcatatttgctctggctaatggagcaaaagcgacgggcaggtaaagacgtgcattacgttttcatggatacaggttgtgaacatccaatgacatatcggtttgtcagggaagttgtgaagttctgggatataccgctcaccgtattgcaggttgatatcaacccggagcttggacagccaaatggttatacggtatgggaaccaaaggatattcagacgcgaatgcctgttctgaagccatttatcgatatggtaaagaaatatggcactccatacgtcggcggcgcgttctgcactgacagattaaaactcgttcccttcaccaaatactgtgatgaccatttcgggcgagggaattacaccacgtggattggcatcagagctgatgaaccgaagcggctaaagccaaagcctggaatcagatatcttgctgaactgtcagactttgagaaggaagatatcctcgcatggtggaagcaacaaccattcgatttgcaaataccggaacatctcggtaactgcatattctgcattaaaaaatcaacgcaaaaaatcggacttgcctgcaaagatgaggagggattgcagcgtgtttttaatgaggtcatcacgggatcccatgtgcgtgacggacatcgggaaacgccaaaggagattatgtaccgaggaagaatgtcgctggacggtatcgcgaaaatgtattcagaaaatgattatcaagccctgtatcaggacatggtacgagctaaaagattcgataccggctcttgttctgagtcatgcgaaatatttggagggcagcttgatttcgacttcgggagggaagctgcatgatgcgatgttatcggtgcggtgaatgcaaagaagataaccgcttccgaccaaatcaaccttactggaatcgatggtgtctccggtgtgaaagaacaccaacaggggtgttaccactaccgcaggaaaaggaggacgtgtggcgagacagcgacgaagtatcaccgacataatctgcgaaaactgcaaataccttccaacgaaacgcaccagaaataaacccaagccaatcccaaaagaatctgacgtaaaaaccttcaactacacggctcacctgtgggatatccggtggctaagacgtcgtgcgaggaaaacaaggtgattgaccaaaatcgaagttacgaacaagaaagcgtcgagcgagctttaacgtgcgctaactgcggtcagaagctgcatgtgctggaagttcacgtgtgtgagcactgctgcgcagaactgatgagcgatccgaatagctcgatgcacgaggaagaagatgatggctaaaccagcgcgaagacgatgtaaaaacgatgaatgccgggaatggtttcaccctgcattcgctaatcagtggtggtgctctccagagtgtggaaccaagatagcactcgaacgacgaagtaaagaacgcgaaaaagcggaaaaagcagcagagaagaaacgacgacgagaggagcagaaacagaaagataaacttaagattcgaaaactcgccttaaagccccgcagttactggattaaacaagcccaacaagccgtaaacgccttcatcagagaaagagaccgcgacttaccatgtatctcgtgcggaacgctcacgtctgctcagtgggatgccggacattaccggacaactgctgcggcacctcaactccgatttaatgaacgcaatattcacaagcaatgcgtggtgtgcaaccagcacaaaagcggaaatctcgttccgtatcgcgtcgaactgattagccgcatcgggcaggaagcagtagacgaaatcgaatcaaaccataaccgccatcgctggactatcgaagagtgcaaggcgatcaaggcagagtaccaacagaaactcaaagacctgcgaaatagcagaagtgaggccgcatgacgttctcagtaaaaaccattccagacatgctcgttgaaacatacggaaatcagacagaagtagcacgcagactgaaatgtagtcgcggtacggtcagaaaatacgttgatgataaagacgggaaaatgcacgccatcgtcaacgacgttctcatggttcatcgcggatggagtgaaagagatgcgctattacgaaaaaattgatggcagcaaataccgaaatatttgggtagttggcgatctgcacggatgctacacgaacctgatgaacaaactggatacgattggattcgacaacaaaaaagacctgcttatctcggtgggcgatttggttgatcgtggtgcagagaacgttgaatgcctggaattaatcacattcccctggttcagagctgtacgtggaaaccatgagcaaatgatgattgatggcttatcagagcgtggaaacgttaatcactggctgcttaatggcggtggctggttctttaatctcgattacgacaaagaaattctggctaaagctcttgcccataaagcagatgaacttccgttaatcatcgaactggtgagcaaagataaaaaatatgttatctgccacgccgattatccctttgacgaatacgagtttggaaagccagttgatcatcagcaggtaatctggaaccgcgaacgaatcagcaactcacaaaacgggatcgtgaaagaaatcaaaggcgcggacacgttcatctttggtcatacgccagcagtgaaaccactcaagtttgccaaccaaatgtatatcgataccggcgcagtgttctgcggaaacctaacattgattcaggtacagggagaaggcgcatgagactcgaaagcgtagctaaatttcattcgccaaaaagcccgatgatgagcgactcaccacgggccacggcttctgactctctttccggtactgatgtgatggctgctatggggatggcgcaatcacaagccggattcggtatggctgcattctgcggtaagcacgaactcagccagaacgacaaacaaaaggctatcaactatctgatgcaatttgcacacaaggtatcggggaaataccgtggtgtggcaaagcttgaaggaaatactaaggcaaaggtactgcaagtgctcgcaacattcgcttatgcggattattgccgtagtgccgcgacgccgggggcaagatgcagagattgccatggtacaggccgtgcggttgatattgccaaaacagagctgtgggggagagttgtcgagaaagagtgcggaagatgcaaaggcgtcggctattcaaggatgccagcaagcgcagcatatcgcgctgtgacgatgctaatcccaaaccttacccaacccacctggtcacgcactgttaagccgctgtatgacgctctggtggtgcaatgccacaaagaagagtcaatcgcagacaacattttgaatgcggtcacacgttagcagcatgattgccacggatggcaacatattaacggcatgatattgacttattgaataaaattgggtaaatttgactcaacgatgggttaattcgctcgttgtggtagtgagatgaaaagaggcggcgcttactaccgattccgcctagttggtcacttcgacgtatcgtctggaactccaaccatcgcaggcagagaggtctgcaaaatgcaatcccgaaacagttcgcaggtaatagttagagcctgcataacggtttcgggattttttatatctgcacaacaggtaagagcattgagtcgataatcgtgaagagtcggcgagcctggttagccagtgctctttccgttgtgctgaattaagcgaataccggaagcagaaccggatcaccaaatgcgtacaggcgtcatcgccgcccagcaacagcacaacccaaactgagccgtagccactgtctgtcctgaattcattagtaatagttacgctgcggccttttacacatgaccttcgtgaaagcgggtggcaggaggtcgcgctaacaacctcctgccgttttgcccgtgcatatcggtcacgaacaaatctgattactaaacacagtagcctggatttgttctatcagtaatcgaccttattcctaattaaatagagcaaatccccttattgggggtaagacatgaagatgccagaaaaacatgacctgttggccgccattctcgcggcaaaggaacaaggcatcggggcaatccttgcgtttgcaatggcgtaccttcgcggcagatataatggcggtgcgtttacaaaaacagtaatcgacgcaacgatgtgcgccattatcgcctagttcattcgtgaccttctcgacttcgccggactaagtagcaatctcgcttatataacgagcgtgtttatcggctacatcggtactgactcgattggttcgcttatcaaacgcttcgctgctaaaaaagccggagtagaagatggtagaaatcaataatcaacgtaaggcgttcctcgatatgctggcgtggtcggagggaactgataacggacgtcagaaaaccagaaatcatggttatgacgtcattgtaggcggagagctatttactgattactccgatcaccctcgcaaacttgtcacgctaaacccaaaactcaaatcaacaggctaagactggccgtcgttttacaacacagaaagagtttgtagaaacgcaaaaaggccatccgtcaggggccttctgcttagtttgatgcctggcagttccctactctcgccttccgcttcctcgctcactgactcgctgcgctcggtcgttcggctgcggcgagcggtatcagctcactcaaaggcggtaatacggttatccacagaatcaggggataacgcaggaaagaacatgtgagcaaaaggccagcaaaaggccaggaaccgtaaaaaggccgcgttgctggcgtttttccataggctccgcccccctgacgagcatcacaaaaatcgacgctcaagtcagaggtggcgaaacccgacaggactataaagataccaggcgtttccccctggaagctccctcgtgcgctctcctgttccgaccctgccgcttaccggatacctgtccgcctttctcccttcgggaagcgtggcgctttctcatagctcacgctgtaggtatctcagttcggtgtaggtcgttcgctccaagctgggctgtgtgcacgaaccccccgttcagcccgaccgctgcgccttatccggtaactatcgtcttgagtccaacccggtaagacacgacttatcgccactggcagcagccactggtaacaggattagcagagcgaggtatgtaggcggtgctacagagttcttgaagtggtgggctaactacggctacactagaagaacagtatttggtatctgcgctctgctgaagccagttaccttcggaaaaagagttggtagctcttgatccggcaaacaaaccaccgctggtagcggtggtttttttgtttgcaagcagcagattacgcgcagaaaaaaaggatctcaagaagatcctttgatcttttctacggggtctgacgctcagtggaacgacgcgcgcgtaactcacgttaagggattttggtcatgagcttgcgccgtcccgtcaagtcagcgtaatgctctgct